European Patent Application EP 4 421 172 A1, published August 28, 2024. Title: 衔接体、复合物、单链分子、试剂盒、方法和应用. Applicant: QITAN TECHNOLOGY LTD.,CHENGDU. The sequence listing filed with the application follows.

SEQUENCE LISTING (4 sequences)

SEQ ID NO: 1 - protein, 439 aa, enterobacteria phage T4
GTFDDLTEGQKNAFNIVMKAIKEKKHHVTINGPAGTGKTTLTKFIIEALISTGETGIILAAPTHAAKKILSKLSGKEASTIHSILKINPVTYECNVLFEQKEVPDLAKARVLICDEVSMYDRKLFKILLSTIPPWATIIGIGDNKQIRPVDPGENTAYISPFFTHKDFYQCELTEVKRSNAPIIDVATDVRNGKWIYDKVVDGHGVRGFTGDTALRDFMVNYFSIVKSLDDLFENRVMAFTNKSVDKLNSIIRKKIFETDKDFIVGEIIVMQEPLFKTYKIDGKPVSEIIFNNGQLVRIIEAEYTSTFVKARGVPGEYLIRHWDLTVETYGDDEYYREKIKIISSDEELYKFNLFLGKTCETYKNWNKGGKAPWSDFWDAKSQFSKVKALPASTFHKAQGMSVDRAFIYTPCIHYADVELAQQLLYVGVTRGRYDVFYV

SEQ ID NO: 2 - DNA, 81 bp, synthetic construct
  source 1..81: mol_type = other DNA
gcggagtcaaacggtagaagtcgttttttttttactgctcattcggtcctgctgactactgctcattcggtcctgctgact

SEQ ID NO: 3 - DNA, 23 bp, synthetic construct
  misc_feature 1..23: note = 1
  source 1..23: mol_type = other DNA
cgacttctaccgtttgactccgc

SEQ ID NO: 4 - DNA, 38 bp, synthetic construct
  source 1..38: mol_type = other DNA
gtcagcaggaccgaatgagcagtagtccagcaccgacc